European Patent Application EP 4 124 343 A1, published February 1, 2023. Title: Novel CD47 Monoclonal Antibodies and Uses Thereof. Applicant: I-Mab. Application EP. The sequence listing filed with the application follows.

SEQUENCE LISTING (107 sequences)

SEQ ID NO: 1 - protein, 119 aa, Homo sapiens
QVQLQQSGGGLVQPGGSLRLSCTASGFTFSSYAMSWVRQAPGKGLEWVSAISGSGGSTYYADSVKGRFTISRDNSKNTLYLQMNSLRVEDTAVYYCARYSIGRHTFDHWGQGTLVTVSA

SEQ ID NO: 2 - protein, 111 aa, Homo sapiens
NFMLTQPHSVSESPGKTVTISCTRSSGGIASNFVQWYQQRPGSVPTTVIYRDNQRPSGVPDRFSGSVDSSSNSASLTISGLKTDDEADYYCQSYDDHNHWVFGGGTKLTVL

SEQ ID NO: 3 - protein, 118 aa, Homo sapiens
KVQLVESGGGLVKPGGSLRLSCAASGFTFSNAWMNWVRQAPGKGLEWVGRIKRKTDGETTDYAAPVKGRFSISRDDSKNTLYLQMNSLKTEDTAVYYCAGSNRAFDIWGQGTMVTVSA

SEQ ID NO: 4 - protein, 113 aa, Homo sapiens
DIVMTQSPDSLAVSLGERATINCKSSQSVLYSSNNRNYLAWYQQKPGQPPKLLINQASTRASGVPDRFSGSGSGTEFTLIISSLHAEDVAIYYCQQYYTPPLAFGGGTKLEIK

SEQ ID NO: 5 - protein, 118 aa, Homo sapiens
QVQLQQSGGGLVQPGGSLRLSCAASGFTFSGYAMTWVRQAPGKGLEWVSAITSTGGRTYYADSVKGRFTTSRDNSRNTLYLQMNSLRAEDTAVYYCARESNFRAFDIWGQGTMVTVSA

SEQ ID NO: 6 - protein, 112 aa, Homo sapiens
EIVLTQSPLSLPVTPGEPASISCRSSQSLLHSNGYNYLDWYLQKPGQSPQLLIYLNSNRASGVPDRFSGSGSGTDFTLQISRVEAEDVGVYYCMQALQIPPTFGGGTKVDIK

SEQ ID NO: 7 - protein, 118 aa, Homo sapiens
EVQLVESGGGLVQPGGSLRLSCAASGFTFIDAWMTWVRQAPGKGLEWVSVIYSGGSTYYADSVKGRFTISRDNSKNTLYLQMNSLRAEDTAVYYCARGARGHPGQDYWGQGTLVTVSA

SEQ ID NO: 8 - protein, 112 aa, Homo sapiens
NFMLTQPHSVSESPGKTVTISCTRSSGTIASNFVQWYQQRPGSSPTPVIFENDRRPSGVPDRFSGSIDSSSNSASLTISSLNTEDKADYYCQSYDSSTHGWVFGGGTQLTVL

SEQ ID NO: 9 - protein, 117 aa, Homo sapiens
QVNLRESGGGLVQPGGSLRLSCAASGFTFSDYYMSWIRQAPGGGLEWVSYTSRFGSDTNYADSVKGRFTISRDNVQNSLYLQMNSLRAEDTAVYYCVRDVHNRDAYWGQGTLVTVSA

SEQ ID NO: 10 - protein, 110 aa, Homo sapiens
SYVLTQPPSASGTPGQRVTISCSGSSSNIGGNSVSWYQQLPGTAPKLLIYRNHQRPSGVPDRFSGSKSGTSASLAISGLRSDDEADYYCATWDFSLSGFVFGTGTKVTVL

SEQ ID NO: 11 - protein, 108 aa, Homo sapiens
QVQLVQSGGGLVQPGGSLRLSCAASGFTFSSYAMSWVRQAPGKGLEWVSAISGSGGSTYYADSVKGRFTISRDNSKNTYYCANTDYYDSSSHTPADYWGQGTLVTVSA

SEQ ID NO: 12 - protein, 108 aa, Homo sapiens
ETTLTQSPSSLSASVGDRVTITCRASQDIRNDLDWFQQKPGEAPKRLISAASNLQSGVPSRFSGGGSGSEFTLTIHSLESEDFATYYCQQSYITPPWTFGQGTKLEIK

SEQ ID NO: 13 - protein, 122 aa, Homo sapiens
QVQLQESGGGLVQPGGSLRLSCAASGFTFSSYGMSWVRQAPGKGLEWVSTISGSGSSTNYADSVKGRFTISRDNSKNTLFLQMNSLRAEDTAVYFCAKGRYYYDSLDAFDIWGQGTMVTVSA

SEQ ID NO: 14 - protein, 108 aa, Homo sapiens
EIVLTQSPGTLSLSPGERATLSCRASQEIRTAYLAWYQQKPGQAPRLLIYYASSRATGIPDRFSGSRSGTDFTLTISRLEPEDFAVYSCQQYDTSPPTFGQGTRLEIK

SEQ ID NO: 15 - protein, 122 aa, Homo sapiens
QVQLVESGGGLVQPGGSLRLSCAASGFTFSSYAMSWVRQAPGKGLEWVSAISGTGGSTYYADSVKGRFTISRDNSKNTLYLQMNSLRAEDTAAYYCAKDKWSSWPTYYFDYWGQGTLVTVSA

SEQ ID NO: 16 - protein, 110 aa, Homo sapiens
NFMLTQPHSVSESPGKTVTISCTRSSGSIASNYVQWYQQRPGSSPTTVIYEDNQRPSGVPDRFSGSIDSSSNSASLTISGLKTEDEADYYCQSYDSSNVIFGGGTKVTVL

SEQ ID NO: 17 - protein, 122 aa, Homo sapiens
QVQLQVSGGGLVQPGGSLRLSCAASGFTFSSYSMAWVRQAPGKGLEWVAAVSNSGVETYYADSVKGRFTISRDNSKNTLYLQMNSLRAEDTAVYYCAKRTRQLLTPREFDYWGQGTLVTVLA

SEQ ID NO: 18 - protein, 107 aa, Homo sapiens
ETTLTQSPSSVSASVGDRVTLTCRASQDITRWLAWYQQKPGKAPKLLIYDASSLQSGVPSRFSGSGSGTDFTLTISSLQPEDFATYYCQQGSSVPFTFGGGTKVEIK

SEQ ID NO: 19 - protein, 117 aa, Homo sapiens
QVNLRESGGGLIQPGGSLRLSCAASGFTFTNYAMSWVRQAPGKGLEWVSSVSSAGGSTYYADSVKGRFTISRDNAKNSLYLQMNSLRAEDTAVYYCARRVNRAFDLWGRGTLVTVSA

SEQ ID NO: 20 - protein, 110 aa, Homo sapiens
DVVMTQSPGTLSLSPGERATLSCRASQSVSSSYLAWYQQKPGQAPRLLIYGASSRATGIPDRFSGSGSGTDFTLTISRLEPEDFAVYYCQQYGSSPPMYTFGQGTKLEIK

SEQ ID NO: 21 - protein, 121 aa, Homo sapiens
QVQLQESGGGLVQPGGSLRLSCAASGFTFSNAWMSWVRQAPGKGLVWVGRIKSKTDGGTTDYAAPVKGRFTISRDDSKNTLYLQMNSLKTEDTAVYYCTTDKSYGYTFDYWGQGTLVTVSA

SEQ ID NO: 22 - protein, 110 aa, Homo sapiens
SYVLTQPPSASGTPGQRVTISCSGSGSNIGSNSVHWYQQLPGTAPKLLIYTNNQRPSGVPDRFSGSKSGISASLAISGLQSEDEAVYYCATWDDRLSGPVFAAGTKLTVL

SEQ ID NO: 23 - protein, 119 aa, Homo sapiens
QVNLRESGGGLVKPGGSLRLSCAASGFTFSSYWMHWVRQAPGKGLEWVSAISGSGAGTYYPDSVKGRFTISRDNSKNTLYLQMNSLRAEDTAVYYCARDRSLSFGFDIWGQGTLVSVSG

SEQ ID NO: 24 - protein, 110 aa, Homo sapiens
NFMLTQPHSVSGSPGKTVTISCTRSSGSIGSTYVQWYQQRPGSPPTTVIYKDDQRPSGVPDRFSGSIDGSSNSASLTISGLETEDEADYYCQSSDTSNLVFGGGTKVTVL

SEQ ID NO: 25 - protein, 121 aa, Homo sapiens
QVQLQQSGGGLVQPGGSLRLSCAAPGFTFSRYWMSWVRQAPGKGLEWVANIKGDGSQTYYADSVKGRFTISRDNAMKTVYLQMNSLRAEDTAIYYCAKGAAYHINSWLDPWGQGTLVTVSA

SEQ ID NO: 26 - protein, 108 aa, Homo sapiens
ETTLTQSPGTLSVSPGERVTLSCRASQSISGNYLAWYQQRPGQAPRLLIYGAFRRATGIPDRFSGSGSGTDFTLTITRLEPEDFATYYCQHYNNFPHTFGAGTKVDIK

SEQ ID NO: 27 - protein, 118 aa, Homo sapiens
KVQLVESGGGLVKPGGSLRLSCAASGITFKHAWMNWVRQAPGKGLEWVGRIKRKTDGETTDYAAPVKGRFSISRDDSKNTLYLQMNSLKTEDTAVYYCAGSNRAFDIWGQGTMVTVSA

SEQ ID NO: 28 - protein, 113 aa, Homo sapiens
DIVMTQSPDSLAVSLGERATINCKSSQSVLYQVNNRNYLAWYQQKPGQPPKLLINQASTRASGVPDRFSGSGSGTEFTLIISSLQAEDVAIYYCQQYYTPPLAFGGGTKLEIK

SEQ ID NO: 29 - protein, 118 aa, Homo sapiens
KVQLVESGGGLVKPGGSLRLSCAASGFTFNNAWMNWVRQAPGKGLEWVGRIKRKTDGETTDYAAPVKGRFSISRDDSKNTLYLQMNSLKTEDTAVYYCAGSNRAFDIWGQGTMVTVSA

SEQ ID NO: 30 - protein, 113 aa, Homo sapiens
DIVMTQSPDSLAVSLGERATINCKSSQTVLYPLNNRNYLAWYQQKPGQPPKLLINQASTRASGVPDRFSGSGSGTEFTLIISSLQAEDVAIYYCQQYYTPPLAFGGGTKLEIK

SEQ ID NO: 31 - protein, 118 aa, Homo sapiens
KVQLVESGGGLVKPGGSLRLSCAASGLTFERAWMNWVRQAPGKGLEWVGRIKRKTDGETTDYAAPVKGRFSISRDDSKNTLYLQMNSLKTEDTAVYYCAGSNRAFDIWGQGTMVTVSA

SEQ ID NO: 32 - protein, 113 aa, Homo sapiens
DIVMTQSPDSLAVSLGERATINCKSSQSVLYAGNNRNYLAWYQQKPGQPPKLLINQASTRASGVPDRFSGSGSGTEFTLIISSLQAEDVAIYYCQQYYTPPLAFGGGTKLEIK

SEQ ID NO: 33 - protein, 118 aa, Homo sapiens
KVQLVESGGGLVKPGGSLRLSCAASGFTFPNAWMNWVRQAPGKGLEWVGRIKRKTDGETTDYAAPVKGRFSISRDDSKNTLYLQMNSLKTEDTAVYYCAGSNRAFDIWGQGTMVTVSA

SEQ ID NO: 34 - protein, 113 aa, Homo sapiens
DIVMTQSPDSLAVSLGERATINCKSSQSVLYPGNNRNYLAWYQQKPGQPPKLLINQASTRASGVPDRFSGSGSGTEFTLIISSLQAEDVAIYYCQQYYTPPLAFGGGTKLEIK

SEQ ID NO: 35 - protein, 118 aa, Homo sapiens
KVQLVESGGGLVKPGGSLRLSCAASGLTFGNAWMNWVRQAPGKGLEWVGRIKRKTDGETTDYAAPVKGRFSISRDDSKNTLYLQMNSLKTEDTAVYYCAGSNRAFDIWGQGTMVTVSA

SEQ ID NO: 36 - protein, 113 aa, Homo sapiens; identical to SEQ ID NO: 34

SEQ ID NO: 37 - protein, 118 aa, Homo sapiens
KVQLVESGGGLVKPGGSLRLSCAASGFTFSNAWMNWVRQAPGKGLEWVGRIKRKTDGETTDYAAPVKGRFSISRDDSKNTLYLQMNSLKTEDTAVYYCAGGNHSSDIWGQGTMVTVSA

SEQ ID NO: 38 - protein, 113 aa, Homo sapiens
DIVMTQSPDSLAVSLGERATINCKSSQSVLYSSNNRNYLAWYQQKPGQPPKLLINQASTRASGVPDRFSGSGSGTEFTLIISSLQAEDVAIYYCQQYYTPPLAFGGGTKLEIK

SEQ ID NO: 39 - protein, 118 aa, Homo sapiens
KVQLVESGGGLVKPGGSLRLSCAASGFTFSNAWMNWVRQAPGKGLEWVGRIKRKTDGETTDYAAPVKGRFSISRDDSKNTLYLQMNSLKTEDTAVYYCAGGAHSSDIWGQGTMVTVSA

SEQ ID NO: 40 - protein, 113 aa, Homo sapiens; identical to SEQ ID NO: 38

SEQ ID NO: 41 - protein, 118 aa, Homo sapiens
KVQLVESGGGLVKPGGSLRLSCAASGFTFSNAWMNWVRQAPGKGLEWVGRIKRKTDGETTDYAAPVKGRFSISRDDSKNTLYLQMNSLKTEDTAVYYCAGGQHSSDIWGQGTMVTVSA

SEQ ID NO: 42 - protein, 113 aa, Homo sapiens; identical to SEQ ID NO: 38

SEQ ID NO: 43 - protein, 118 aa, Homo sapiens
KVQLVESGGGLVKPGGSLRLSCAASGFTFSNAWMNWVRQAPGKGLEWVGRIKRKTDGETTDYAAPVKGRFSISRDDSKNTLYLQMNSLKTEDTAVYYCAGSAYAFDAWGQGTMVTVSA

SEQ ID NO: 44 - protein, 113 aa, Homo sapiens; identical to SEQ ID NO: 38

SEQ ID NO: 45 - protein, 118 aa, Homo sapiens
KVQLVESGGGLVKPGGSLRLSCAASGFTFSNAWMNWVRQAPGKGLEWVGRIKRKTDGETTDYAAPVKGRFSISRDDSKNTLYLQMNSLKTEDTAVYYCAGSAYAFDSWGQGTMVTVSA

SEQ ID NO: 46 - protein, 113 aa, Homo sapiens; identical to SEQ ID NO: 38

SEQ ID NO: 47 - protein, 118 aa, Homo sapiens
KVQLVESGGGLVKPGGSLRLSCAASGFTFSNAWMNWVRQAPGKGLEWVGRIKRKTDGETTDYAAPVKGRFSISRDDSKNTLYLQMNSLKTEDTAVYYCAGSDRASDKWGQGTMVTVSA

SEQ ID NO: 48 - protein, 113 aa, Homo sapiens; identical to SEQ ID NO: 38

SEQ ID NO: 49 - protein, 118 aa, Homo sapiens
KVQLVESGGGLVKPGGSLRLSCAASGFTFSNAWMNWVRQAPGKGLEWVGRIKRKTDGETTDYAAPVKGRFSISRDDSKNTLYLQMNSLKTEDTAVYYCAGSAYAFDTWGQGTMVTVSA

SEQ ID NO: 50 - protein, 113 aa, Homo sapiens; identical to SEQ ID NO: 38

SEQ ID NO: 51 - protein, 118 aa, Homo sapiens
KVQLVESGGGLVKPGGSLRLSCAASGFTFSNAWMNWVRQAPGKGLEWVGRIKRKTDGETTDYAAPVKGRFSISRDDSKNTLYLQMNSLKTEDTAVYYCAGGNHSQDIWGQGTMVTVSA

SEQ ID NO: 52 - protein, 113 aa, Homo sapiens; identical to SEQ ID NO: 38

SEQ ID NO: 53 - protein, 118 aa, Homo sapiens
KVQLVESGGGLVKPGGSLRLSCAASGFTFSNAWMNWVRQAPGKGLEWVGRIKRKTDGETTDYAAPVKGRFSISRDDSKNTLYLQMNSLKTEDTAVYYCAGGQHSQDIWGQGTMVTVSA

SEQ ID NO: 54 - protein, 113 aa, Homo sapiens; identical to SEQ ID NO: 38

SEQ ID NO: 55 - protein, 118 aa, Homo sapiens
KVQLVESGGGLVKPGGSLRLSCAASGFTFSNAWMNWVRQAPGKGLEWVGRIKRKTDGETTDYAAPVKGRFSISRDDSKNTLYLQMNSLKTEDTAVYYCAGGAHSQDIWGQGTMVTVSA

SEQ ID NO: 56 - protein, 113 aa, Homo sapiens; identical to SEQ ID NO: 38

SEQ ID NO: 57 - protein, 118 aa, Homo sapiens; identical to SEQ ID NO: 3

SEQ ID NO: 58 - protein, 113 aa, Homo sapiens
DIVMTQSPDSLAVSLGERATINCKSSQSVLYSSNNRNYLAWYQQKPGQPPKLLINQASTRASGVPDRFSGSGSGTEFTLIISSLQAEDVAIYYCQQYLTPPLAFGGGTKLEIK

SEQ ID NO: 59 - protein, 118 aa, Homo sapiens; identical to SEQ ID NO: 3

SEQ ID NO: 60 - protein, 113 aa, Homo sapiens
DIVMTQSPDSLAVSLGERATINCKSSQSVLYSSNNRNYLAWYQQKPGQPPKLLINQASTRASGVPDRFSGSGSGTEFTLIISSLQAEDVAIYYCQQYLRPPLNFGGGTKLEIK

SEQ ID NO: 61 - protein, 118 aa, Homo sapiens; identical to SEQ ID NO: 3

SEQ ID NO: 62 - protein, 113 aa, Homo sapiens
DIVMTQSPDSLAVSLGERATINCKSSQSVLYSSNNRNYLAWYQQKPGQPPKLLINQASTRASGVPDRFSGSGSGTEFTLIISSLQAEDVAIYYCQQYLTPPLNFGGGTKLEIK

SEQ ID NO: 63 - protein, 118 aa, Homo sapiens; identical to SEQ ID NO: 3

SEQ ID NO: 64 - protein, 113 aa, Homo sapiens
DIVMTQSPDSLAVSLGERATINCKSSQSVLYSSNNRNYLAWYQQKPGQPPKLLINQASTRASGVPDRFSGSGSGTEFTLIISSLQAEDVAIYYCQNYLTPPLSFGGGTKLEIK

SEQ ID NO: 65 - protein, 118 aa, Homo sapiens; identical to SEQ ID NO: 3

SEQ ID NO: 66 - protein, 113 aa, Homo sapiens
DIVMTQSPDSLAVSLGERATINCKSSQSVLYSSNNRNYLAWYQQKPGQPPKLLINQASTRASGVPDRFSGSGSGTEFTLIISSLQAEDVAIYYCQQYLKAPLAFGGGTKLEIK

SEQ ID NO: 67 - protein, 118 aa, Homo sapiens; identical to SEQ ID NO: 3

SEQ ID NO: 68 - protein, 113 aa, Homo sapiens
DIVMTQSPDSLAVSLGERATINCKSSQSVLYSSNNRNYLAWYQQKPGQPPKLLINQASTRASGVPDRFSGSGSGTEFTLIISSLQAEDVAIYYCQQYLNAPLHFGGGTKLEIK

SEQ ID NO: 69 - protein, 118 aa, Homo sapiens; identical to SEQ ID NO: 3

SEQ ID NO: 70 - protein, 113 aa, Homo sapiens
DIVMTQSPDSLAVSLGERATINCKSSQSVLYSSNNRNYLAWYQQKPGQPPKLLINQASTRASGVPDRFSGSGSGTEFTLIISSLQAEDVAIYYCQQYLEAPLVFGGGTKLEIK

SEQ ID NO: 71 - protein, 118 aa, Homo sapiens; identical to SEQ ID NO: 3

SEQ ID NO: 72 - protein, 113 aa, Homo sapiens
DIVMTQSPDSLAVSLGERATINCKSSQSVLYSSNNRNYLAWYQQKPGQPPKLLINQASTRASGVPDRFSGSGSGTEFTLIISSLQAEDVAIYYCQQYLKAPLHFGGGTKLEIK

SEQ ID NO: 73 - protein, 118 aa, Homo sapiens; identical to SEQ ID NO: 3

SEQ ID NO: 74 - protein, 113 aa, Homo sapiens
DIVMTQSPDSLAVSLGERATINCKSSQSVLYSSNNRNYLAWYQQKPGQPPKLLINQASTRASGVPDRFSGSGSGTEFTLIISSLQAEDVAIYYCQRLIAPPFTFGGGTKLEIK

SEQ ID NO: 75 - protein, 118 aa, Homo sapiens; identical to SEQ ID NO: 3

SEQ ID NO: 76 - protein, 113 aa, Homo sapiens
DIVMTQSPDSLAVSLGERATINCKSSQSVLYSSNNRNYLAWYQQKPGQPPKLLINQASTRASGVPDRFSGSGSGTEFTLIISSLQAEDVAIYYCQNYLTPPLAFGGGTKLEIK

SEQ ID NO: 77 - DNA, 360 bp, Homo sapiens
caggtccaactggtgcagtctggggctgaagtgaagaagcctgggtcttcagtgaaggtgtcctgcaaggcttctggctacaccttcagcagctactatatgcactgggtgaggcaggctcctggacaaggccttgagtggatgggagagattaatcccaacaatgcccgtattaacttcaatgaaaagttcaagaccagggtcacactcactgtggacaaatccaccagcacagcatacatggagctcagcagcctgagatctgaggacaccgcggtctattactgtaccagaggatactataggtacggggcctggtttggttactggggccaagggactctggtcactgtctcttca

SEQ ID NO: 78 - DNA, 321 bp, Homo sapiens
gatatccagatgacacagtctccatcctccctgtctgcctctgtgggagacagagtcaccatcacttgcagggcaagtcaggacattagcgattatttgaactggtatcaacagaaaccaggcaaggctcctaaactcctgatctactacatatcaagattacactcaggagtcccatcacgcttcagtggcagtgggtctggaacagattatactctcaccattagctccctgcagccagaagattttgccacttactattgccaacagggtcatacacttccgtggaccttcggtggaggcaccaaggtggaaatcaaa

SEQ ID NO: 79 - DNA, 357 bp, Homo sapiens
caggtacagctgcagcagtcagggggaggcttggtacagcctggggggtccctaagactctcctgtacagcctctggattcacctttagcagctatgccatgagctgggtccgccaggctccagggaaggggctggagtgggtctcagcaattagtggtagtggtggtagcacatactacgcagactccgtgaagggccggttcaccatctccagagacaattccaagaacacgctgtatctgcaaatgaacagcctgagagtcgaggacacggccgtatattactgtgcgagatatagtattggtagacacacctttgaccactggggccagggcaccctggtcaccgtctcggcc

SEQ ID NO: 80 - DNA, 354 bp, Homo sapiens
aaggtgcagctggtggagtctgggggaggcttggtaaagcctggggggtcccttagactctcctgtgcagcctctggtttcactttcagtaacgcctggatgaactgggtccgccaggctccagggaaggggctggagtgggtcggccgtattaaaaggaaaactgatggtgagacaacagactacgctgcacccgtgaaaggcagattcagcatctcaagagatgattcaaaaaacaccctgtatctgcaaatgaacagcttgaaaaccgaggacacagccgtgtattactgcgctggcagtaaccgagcttttgatatctggggccaagggacaatggtcaccgtctctgcc

SEQ ID NO: 81 - DNA, 354 bp, Homo sapiens
caggtacagctgcagcagtcagggggaggcttggtacagcctggggggtccctgagactctcctgtgcagcctctggattcacctttagcggctatgccatgacttgggtccgccaggctccagggaaggggctggagtgggtctcagctattacttctactggtggtcgcacatactacgcagactccgtgaagggccggttcaccacctccagagacaattccaggaacacgttgtatctgcaaatgaacagcctgagagccgaagacacggccgtatattactgtgcgagagagtcaaacttcagggcttttgatatctggggccaagggacaatggtcaccgtctctgcc

SEQ ID NO: 82 - DNA, 354 bp, Homo sapiens
gaggtgcagctggtggagtctgggggaggcttggtacagcctggggggtcccttagactctcctgtgcagcctctggattcactttcattgacgcctggatgacctgggtccgccaggctccagggaaggggctggagtgggtctcagttatttatagcggtggtagcacatactacgcagactccgtgaagggcagattcaccatctccagagacaattccaagaacacgctgtatctgcaaatgaacagcctgagagccgaggacacggccgtatattactgtgcgagaggggctaggggccatcccgggcaggactactgggggcagggcaccctggtcaccgtctcggcc

SEQ ID NO: 83 - DNA, 351 bp, Homo sapiens
caggtcaacttaagggagtctgggggaggcttggtacagcctggcgggtccctgagactctcctgtgcagcctctggattcaccttcagtgactactacatgagctggatccgccaggctccagggggggggctggagtgggtttcatacactagtcgttttggtagtgacacaaactacgcagactctgtgaagggccgattcaccatctccagagacaacgtccagaactcactatatctgcaaatgaacagcctgagggccgaggacacggctgtttattactgtgtgagagatgtacataacagggatgcctactggggccagggcaccctggtcaccgtctcggcc

SEQ ID NO: 84 - DNA, 369 bp, Homo sapiens
caggtgcagctggtgcagtctgggggaggcttggtacagcctggggggtccctgagactctcctgtgcagcctctggattcacctttagcagctatgccatgagctgggtccgccaggctccagggaaggggctggagtgggtctcagctattagtggtagtggtggtagcacatactacgcagactccgtgaagggccggttcaccatctccagagacaattccaagaacacgctgtatctgcaaatgaacagcctgagagccgaggacacggccgtatattactgtgcgaacacagattactatgatagtagtagccatacccccgctgactactggggccagggcaccctggtcaccgtctcggcc

SEQ ID NO: 85 - DNA, 366 bp, Homo sapiens
caggtgcagctgcaggagtcggggggaggcttggtacagcctggggggtccctgagactctcctgtgcagcctctggattcacctttagtagctatggcatgagctgggtccgccaggctccagggaaagggctggagtgggtctcaactatcagtggcagtggtagtagcacaaactacgcagactccgtgaagggccggttcaccatctccagagacaattccaagaacacgctatttctgcaaatgaacagcctgagagccgaggacacggccgtatatttctgtgcgaaaggccgatattactatgatagtcttgatgcttttgatatctggggccaagggacaatggtcaccgtctctgcc

SEQ ID NO: 86 - DNA, 366 bp, Homo sapiens
caggtacagctggtggagtctgggggaggcttggtacagcctggggggtccctgagactctcctgtgcagcctctggattcacctttagcagctatgccatgagctgggtccgccaggctccagggaaggggctggagtgggtctcagctattagtggtactggtggtagcacatactacgcagactccgtgaagggccggttcaccatctccagagacaattccaagaacacgctgtatctgcaaatgaacagcctgagagccgaggacacggccgcatattactgtgcgaaagataaatggagcagctggcccacttactactttgactactggggccagggaaccctggtcaccgtctcggcc

SEQ ID NO: 87 - DNA, 366 bp, Homo sapiens
caggtgcagctgcaggtgtcggggggaggcttggtacagcctggggggtccctgagactctcctgtgcagcctctggattcaccttcagtagctatagcatggcctgggtccgccaggctccagggaaggggctggagtgggtcgcggctgttagtaatagtggtgttgagacatactacgcagactccgtgaagggccggttcaccatctccagagacaattccaagaacacgctgtatttgcaaatgaacagcctgagagccgaggacacggccgtatattactgtgcgaaacgaactagacaactgctaactccgcgggagtttgactactggggccagggcaccctggtcaccgtcttggcc

SEQ ID NO: 88 - DNA, 351 bp, Homo sapiens
caggtcaacttaagggagtctgggggaggcttgatacagcctggggggtccctgagactctcctgtgcagcctctggattcacctttaccaattatgccatgagctgggtccgccaggctccagggaaggggctggagtgggtctcaagtgttagtagtgctggtggtagtacatactacgcagactccgtgaagggccggttcaccatctccagagacaacgccaagaactcactgtatctgcaaatgaacagcctgagagccgaggacacggctgtttattactgtgcgagacgagtcaatcgggccttcgatctctggggccgtggaaccctggtcaccgtctcggcc

SEQ ID NO: 89 - DNA, 363 bp, Homo sapiens
caggtgcagctgcaggagtcggggggaggcttggtacagcctggggggtcccttagactctcctgtgcagcctctggattcactttcagtaacgcctggatgagctgggtccgccaggctccagggaaggggctggtgtgggttggccgtattaaaagcaaaactgatggtgggacaacagactacgctgcacccgtgaaaggcagattcaccatctcaagagatgattcaaaaaacacgctgtatctgcaaatgaacagcctgaaaaccgaggacacagccgtgtattactgtaccacagataagagctatggttacacatttgactactggggccagggcaccctggtcaccgtctcggcc

SEQ ID NO: 90 - DNA, 357 bp, Homo sapiens
caggtcaacttaagggagtctgggggaggcttggtaaagccgggggggtcccttagactctcctgtgcagcctctggattcaccttcagtagctactggatgcactgggtccgccaagccccagggaaggggctggagtgggtctcagctatcagtggtagtggtgccggcacatactacccagactccgtgaagggccggttcaccatctccagagacaattccaagaacacgctgtatctgcaaatgaacagcctgagagccgaggacacggccgtatattactgtgcgagagatcggtccttatcttttggttttgatatttggggccaaggcaccctggtctccgtctctggc

SEQ ID NO: 91 - DNA, 363 bp, Homo sapiens
caggtacagctgcagcagtcagggggaggcttggtccagccgggggggtcactgagactctcctgtgcagcccctggattcacctttagtagatattggatgagttgggtccgccaggctccagggaagggactggagtgggtggccaacataaagggagatggaagtcagacatactatgcggactctgtgaagggccgattcaccatctccagagacaacgccatgaaaacagtgtatctgcaaatgaacagcctgagagccgaggacacggccatatattactgtgcgaaaggggctgcttatcacattaacagctggctcgacccctggggccagggcaccctggtcaccgtctcggcc

SEQ ID NO: 92 - DNA, 333 bp, Homo sapiens
aattttatgctgactcagccccactctgtgtcggagtctccggggaagacggtaaccatctcctgcacccgcagcagtggcggcattgccagtaactttgtgcagtggtaccagcagcgcccgggcagtgtccccaccactgtgatctatagggataaccaaagaccctctggagtccctgatcggttctctggctccgtcgacagctcctccaattctgcctccctcaccatctctgggctgaagactgacgatgaggctgactattattgtcagtcctatgatgaccacaatcattgggtgttcggcggcgggaccaagctgaccgtccta

SEQ ID NO: 93 - DNA, 339 bp, Homo sapiens
gacatcgtgatgacccagtctccagactccctggctgtgtctctgggcgagagggccaccatcaactgcaagtccagccagagtgttttatacagctccaacaataggaactacctagcttggtaccagcagaaaccaggacagcctcctaagctgctcattaaccaggcatctacccgggcatccggcgtccctgaccgattcagtggcagcgggtctgggacagagttcactctcatcatcagcagcctgcaggctgaagatgtggcgatttattactgtcagcaatattatactcctcccctcgctttcggcggagggaccaagctggagatcaaa

SEQ ID NO: 94 - DNA, 336 bp, Homo sapiens
gaaattgtgttgacgcagtctccactctccctgcccgtcacccctggagagccggcctccatctcctgcaggtctagtcagagcctcctgcacagtaatggatacaactatttggattggtacctgcagaaaccagggcagtctccacagctcctgatctatttgaattctaatcgggcctccggggtccctgacaggttcagtggcagtggatcaggtacagattttacactgcaaatcagcagagtggaggctgaggatgttggggtttactactgtatgcaagctctacaaattcctcccactttcggcggagggaccaaagtggatatcaaa

SEQ ID NO: 95 - DNA, 336 bp, Homo sapiens
aattttatgctgactcagccccactctgtgtcggagtctccgggaaagacggtaaccatctcctgcacccgcagcagtggcaccattgccagcaactttgtgcagtggtatcaacagcgcccgggcagttcgcccaccccagtgatctttgagaatgaccgaagaccctctggggtccctgatcggttctctggctccatcgacagctcctccaattctgcctccctcaccatttcgtcactgaacactgaggacaaggctgactactactgtcagtcctatgatagcagcactcatgggtgggtgtttggcggagggacccagctcaccgtttta

SEQ ID NO: 96 - DNA, 330 bp, Homo sapiens
tcctatgtgctgactcagccaccctcagcgtctgggacccccgggcagagggtcaccatctcttgttctggaagcagctccaacatcggcggtaattctgtatcctggtaccagcaactcccaggaacggcccccaagctcctcatctataggaatcatcagcggccctcaggggtccctgaccgattctctggctccaagtctggcacctcagcctccctggccatcagtgggctccggtccgacgacgaggctgattattattgtgcaacatgggatttcagcctgagtggttttgtcttcggaactgggaccaaggtcaccgtccta

SEQ ID NO: 97 - DNA, 324 bp, Homo sapiens
gaaactacactcacgcagtctccatcctccctgtctgcatctgtaggagacagagtcaccatcacttgccgggccagtcaggacatcagaaatgatttagactggtttcaacaaaaaccaggcgaagcccctaaacgcctgatctctgctgcatctaatttgcagagtggggtcccctcacgattcagcggcggtggctctggctccgaattcactctcacaatccacagcctggagtctgaagattttgcaacttactactgtcaacagagttacattacccctccttggacgttcggccaagggaccaagctggagatcaaa

SEQ ID NO: 98 - DNA, 324 bp, Homo sapiens
gaaattgtgttgacgcagtctccaggcaccctgtctttgtctccaggggaaagagccaccctctcctgcagggccagtcaggaaattaggaccgcctacttagcctggtaccagcagaaacctggccaggctcccaggctcctcatctattatgcatccagcagggccactggcatcccagacaggttcagcggcagtaggtctgggacagacttcactctcaccatcagcagactggagcctgaagattttgcagtgtattcctgtcagcagtatgatacctcacctcccaccttcggccaagggacacgactggagattaaa

SEQ ID NO: 99 - DNA, 330 bp, Homo sapiens
aattttatgctgactcagccccactctgtgtcggagtctccggggaagacggtaaccatctcctgcacccgcagcagtggcagcattgccagcaactatgtgcagtggtaccaacagcgcccgggcagttcccccaccactgtgatctatgaggataaccaaagaccctctggggtccctgatcggttctctggctccatcgacagctcctccaactctgcctccctcaccatctctggactgaagactgaggacgaggctgactactactgtcagtcttatgatagcagcaatgtgatattcggcggagggaccaaggtcaccgtccta

SEQ ID NO: 100 - DNA, 321 bp, Homo sapiens
gaaactacactcacgcagtctccatcttccgtgtctgcatctgtaggagacagagtcaccctcacttgtcgggcgagtcaggatatcacaaggtggttagcctggtatcagcagaaaccagggaaagcccctaagctcctgatctatgatgcatccagtttgcaaagtggggtcccatcaagattcagcggcagtggatctgggacagatttcactctcaccatcagcagtctgcaacctgaagattttgcaacttactactgtcaacagggttccagtgttcctttcactttcggcggagggaccaaggtggagatcaaa

SEQ ID NO: 101 - DNA, 330 bp, Homo sapiens
gatgttgtgatgactcagtctccaggcaccctgtctttgtctccaggggaaagagccaccctctcctgcagggccagtcagagtgttagcagcagctacttagcctggtaccaacagaaacctggccaggctcccaggctcctcatctatggtgcatccagcagggccactggcatcccagacaggttcagtggcagtgggtctgggacagacttcactctcaccatcagcagactggagcctgaagattttgcagtgtattactgtcagcagtatggtagctcacctcctatgtacacttttggccaggggaccaagctggagatcaaa

SEQ ID NO: 102 - DNA, 330 bp, Homo sapiens
tcctatgtgctgactcagccaccctcagcgtctgggacccccgggcagagggtcaccatctcttgttctggaagtggctccaacatcggaagtaattctgttcactggtaccagcaactcccaggaacggcccccaaactcctcatctatactaataatcagcggccctcaggggtccctgaccgattctctggctccaagtctggcatttcagcctccctggctatcagtgggctccagtctgaggatgaggctgtttattactgtgcaacgtgggatgacagactgagtggtccggtgttcgccgcagggaccaagctgaccgtccta

SEQ ID NO: 103 - DNA, 330 bp, Homo sapiens
aattttatgctgactcagccccactctgtgtcggggtctccggggaagacggtaaccatctcctgcacccgcagcagtggcagcattggcagcacctatgtgcagtggtaccaacagcgcccgggcagtccccccaccactgtgatctataaggatgaccaaagaccctctggggtccctgatcggttctctggctccatcgacggctcctccaactctgcctccctcaccatctctggactggagactgaggacgaggctgactactactgtcagtcttctgataccagcaatctggtcttcggcggagggaccaaggtcaccgtccta

SEQ ID NO: 104 - DNA, 324 bp, Homo sapiens
gaaactacactcacgcagtctccaggcaccctgtctgtttctccgggggaaagagttaccctctcctgcagggccagtcagagtattagcggtaattacttagcctggtaccagcagagacctggccaggctcccaggctcctcatctatggggcattcaggagggccactggcatcccagacaggttcagtggcagtgggtctgggacagacttcactctcaccatcaccagactggagcctgaagattttgcaacttattactgccaacactataataatttcccccacactttcggcgcagggaccaaagtggatatcaaa

SEQ ID NO: 105 - protein, 120 aa, Homo sapiens
QVQLVQSGAEVKKPGSSVKVSCKASGYTFSSYYMHWVRQAPGQGLEWMGEINPNNARINFNEKFKTRVTLTVDKSTSTAYMELSSLRSEDTAVYYCTRGYYRYGAWFGYWGQGTLVTVSS

SEQ ID NO: 106 - protein, 107 aa, Homo sapiens
DIQMTQSPSSLSASVGDRVTITCRASQDISDYLNWYQQKPGKAPKLLIYYISRLHSGVPSRFSGSGSGTDYTLTISSLQPEDFATYYCQQGHTLPWTFGGGTKVEIK

SEQ ID NO: 107 - protein, 123 aa, Homo sapiens
QLLFNKTKSVEFTFCNDTVVIPCFVTNMEAQNTTEVYVKWKFKGRDIYTFDGALNKSTVPTDFSSAKIEVSQLLKGDASLKMDKSDAVSHTGNYTCEVTELTREGETIIELKYRVVSWFSPNE